European Patent Specification EP 3 981 884 B1, published August 9, 2023. Title: SINGLE CELL WHOLE GENOME LIBRARIES FOR METHYLATION SEQUENCING. Applicant: OREGON HEALTH & SCIENCE UNIVERSITY ILLUMINA, INC. The sequence listing filed with the application follows.

SEQUENCE LISTING (132 sequences)

SEQ ID NO: 1 - DNA, 19 bp, Artificial Sequence
  source: /note="Description of Artificial Sequence: Synthetic oligonucleotide"
ctgtctcttatacacatct

SEQ ID NO: 2 - DNA, 60 bp, Artificial Sequence
  source: /note="Description of Artificial Sequence: Synthetic oligonucleotide"
ggtgtagtgggtttgggttaagaggaatggtagagagggtgagatgtgtataagagacag

SEQ ID NO: 3 - DNA, 60 bp, Artificial Sequence
  source: /note="Description of Artificial Sequence: Synthetic oligonucleotide"
ggtgtagtgggtttggagtaggaagattggtagagagggtgagatgtgtataagagacag

SEQ ID NO: 4 - DNA, 60 bp, Artificial Sequence
  source: /note="Description of Artificial Sequence: Synthetic oligonucleotide"
ggtgtagtgggtttgggaattaggtgttggtagagagggtgagatgtgtataagagacag

SEQ ID NO: 5 - DNA, 60 bp, Artificial Sequence
  source: /note="Description of Artificial Sequence: Synthetic oligonucleotide"
ggtgtagtgggtttggggagattaatgtggtagagagggtgagatgtgtataagagacag

SEQ ID NO: 6 - DNA, 60 bp, Artificial Sequence
  source: /note="Description of Artificial Sequence: Synthetic oligonucleotide"
ggtgtagtgggtttggtattgtggaattggtagagagggtgagatgtgtataagagacag

SEQ ID NO: 7 - DNA, 60 bp, Artificial Sequence
  source: /note="Description of Artificial Sequence: Synthetic oligonucleotide"
ggtgtagtgggtttggatatagatgattggtagagagggtgagatgtgtataagagacag

SEQ ID NO: 8 - DNA, 60 bp, Artificial Sequence
  source: /note="Description of Artificial Sequence: Synthetic oligonucleotide"
ggtgtagtgggtttgggtaagaggaattggtagagagggtgagatgtgtataagagacag

SEQ ID NO: 9 - DNA, 60 bp, Artificial Sequence
  source: /note="Description of Artificial Sequence: Synthetic oligonucleotide"
ggtgtagtgggtttgggagagttattgtggtagagagggtgagatgtgtataagagacag

SEQ ID NO: 10 - DNA, 60 bp, Artificial Sequence
  source: /note="Description of Artificial Sequence: Synthetic oligonucleotide"
ggtgtagtgggtttggagttagtgtgatggtagagagggtgagatgtgtataagagacag

SEQ ID NO: 11 - DNA, 60 bp, Artificial Sequence
  source: /note="Description of Artificial Sequence: Synthetic oligonucleotide"
ggtgtagtgggtttgggatatagaatttggtagagagggtgagatgtgtataagagacag

SEQ ID NO: 12 - DNA, 60 bp, Artificial Sequence
  source: /note="Description of Artificial Sequence: Synthetic oligonucleotide"
ggtgtagtgggtttggaaggaagtgaatggtagagagggtgagatgtgtataagagacag

SEQ ID NO: 13 - DNA, 60 bp, Artificial Sequence
  source: /note="Description of Artificial Sequence: Synthetic oligonucleotide"
ggtgtagtgggtttggaataaggaaggtggtagagagggtgagatgtgtataagagacag

SEQ ID NO: 14 - DNA, 60 bp, Artificial Sequence
  source: /note="Description of Artificial Sequence: Synthetic oligonucleotide"
ggtgtagtgggtttgggtatggatatatggtagagagggtgagatgtgtataagagacag

SEQ ID NO: 15 - DNA, 60 bp, Artificial Sequence
  source: /note="Description of Artificial Sequence: Synthetic oligonucleotide"
ggtgtagtgggtttggttagataatgatggtagagagggtgagatgtgtataagagacag

SEQ ID NO: 16 - DNA, 60 bp, Artificial Sequence
  source: /note="Description of Artificial Sequence: Synthetic oligonucleotide"
ggtgtagtgggtttggggtgttgtaattggtagagagggtgagatgtgtataagagacag

SEQ ID NO: 17 - DNA, 60 bp, Artificial Sequence
  source: /note="Description of Artificial Sequence: Synthetic oligonucleotide"
ggtgtagtgggtttgggaagtggagagtggtagagagggtgagatgtgtataagagacag

SEQ ID NO: 18 - DNA, 60 bp, Artificial Sequence
  source: /note="Description of Artificial Sequence: Synthetic oligonucleotide"
ggtgtagtgggtttggttgagtggtagtggtagagagggtgagatgtgtataagagacag

SEQ ID NO: 19 - DNA, 60 bp, Artificial Sequence
  source: /note="Description of Artificial Sequence: Synthetic oligonucleotide"
ggtgtagtgggtttgggataatggtgatggtagagagggtgagatgtgtataagagacag

SEQ ID NO: 20 - DNA, 60 bp, Artificial Sequence
  source: /note="Description of Artificial Sequence: Synthetic oligonucleotide"
ggtgtagtgggtttgggtgttaatggatggtagagagggtgagatgtgtataagagacag

SEQ ID NO: 21 - DNA, 60 bp, Artificial Sequence
  source: /note="Description of Artificial Sequence: Synthetic oligonucleotide"
ggtgtagtgggtttggtaggaatggtgtggtagagagggtgagatgtgtataagagacag

SEQ ID NO: 22 - DNA, 60 bp, Artificial Sequence
  source: /note="Description of Artificial Sequence: Synthetic oligonucleotide"
ggtgtagtgggtttggatgtatggatatggtagagagggtgagatgtgtataagagacag

SEQ ID NO: 23 - DNA, 60 bp, Artificial Sequence
  source: /note="Description of Artificial Sequence: Synthetic oligonucleotide"
ggtgtagtgggtttggtgattgttggttggtagagagggtgagatgtgtataagagacag

SEQ ID NO: 24 - DNA, 60 bp, Artificial Sequence
  source: /note="Description of Artificial Sequence: Synthetic oligonucleotide"
ggtgtagtgggtttggaagagaattattggtagagagggtgagatgtgtataagagacag

SEQ ID NO: 25 - DNA, 60 bp, Artificial Sequence
  source: /note="Description of Artificial Sequence: Synthetic oligonucleotide"
ggtgtagtgggtttggaatggttggtatggtagagagggtgagatgtgtataagagacag

SEQ ID NO: 26 - DNA, 60 bp, Artificial Sequence
  source: /note="Description of Artificial Sequence: Synthetic oligonucleotide"
ggtgtagtgggtttggggttaattgagtggtagagagggtgagatgtgtataagagacag

SEQ ID NO: 27 - DNA, 60 bp, Artificial Sequence
  source: /note="Description of Artificial Sequence: Synthetic oligonucleotide"
ggtgtagtgggtttgggtataatagtttggtagagagggtgagatgtgtataagagacag

SEQ ID NO: 28 - DNA, 60 bp, Artificial Sequence
  source: /note="Description of Artificial Sequence: Synthetic oligonucleotide"
ggtgtagtgggtttggttagttgaatttggtagagagggtgagatgtgtataagagacag

SEQ ID NO: 29 - DNA, 60 bp, Artificial Sequence
  source: /note="Description of Artificial Sequence: Synthetic oligonucleotide"
ggtgtagtgggtttggttggtgaaggttggtagagagggtgagatgtgtataagagacag

SEQ ID NO: 30 - DNA, 60 bp, Artificial Sequence
  source: /note="Description of Artificial Sequence: Synthetic oligonucleotide"
ggtgtagtgggtttggttaatattgaatggtagagagggtgagatgtgtataagagacag

SEQ ID NO: 31 - DNA, 60 bp, Artificial Sequence
  source: /note="Description of Artificial Sequence: Synthetic oligonucleotide"
ggtgtagtgggtttgggttagaattggtggtagagagggtgagatgtgtataagagacag

SEQ ID NO: 32 - DNA, 60 bp, Artificial Sequence
  source: /note="Description of Artificial Sequence: Synthetic oligonucleotide"
ggtgtagtgggtttgggttattaattatggtagagagggtgagatgtgtataagagacag

SEQ ID NO: 33 - DNA, 60 bp, Artificial Sequence
  source: /note="Description of Artificial Sequence: Synthetic oligonucleotide"
ggtgtagtgggtttgggattggtaagatggtagagagggtgagatgtgtataagagacag

SEQ ID NO: 34 - DNA, 60 bp, Artificial Sequence
  source: /note="Description of Artificial Sequence: Synthetic oligonucleotide"
ggtgtagtgggtttggtgaagtattgttggtagagagggtgagatgtgtataagagacag

SEQ ID NO: 35 - DNA, 60 bp, Artificial Sequence
  source: /note="Description of Artificial Sequence: Synthetic oligonucleotide"
ggtgtagtgggtttgggatggattatgtggtagagagggtgagatgtgtataagagacag

SEQ ID NO: 36 - DNA, 60 bp, Artificial Sequence
  source: /note="Description of Artificial Sequence: Synthetic oligonucleotide"
ggtgtagtgggtttggattagtatatttggtagagagggtgagatgtgtataagagacag

SEQ ID NO: 37 - DNA, 60 bp, Artificial Sequence
  source: /note="Description of Artificial Sequence: Synthetic oligonucleotide"
ggtgtagtgggtttgggtaggtgtggttggtagagagggtgagatgtgtataagagacag

SEQ ID NO: 38 - DNA, 60 bp, Artificial Sequence
  source: /note="Description of Artificial Sequence: Synthetic oligonucleotide"
ggtgtagtgggtttggagttgaatgtatggtagagagggtgagatgtgtataagagacag

SEQ ID NO: 39 - DNA, 60 bp, Artificial Sequence
  source: /note="Description of Artificial Sequence: Synthetic oligonucleotide"
ggtgtagtgggtttggattgtgagatatggtagagagggtgagatgtgtataagagacag

SEQ ID NO: 40 - DNA, 60 bp, Artificial Sequence
  source: /note="Description of Artificial Sequence: Synthetic oligonucleotide"
ggtgtagtgggtttggttgtggtgagttggtagagagggtgagatgtgtataagagacag

SEQ ID NO: 41 - DNA, 60 bp, Artificial Sequence
  source: /note="Description of Artificial Sequence: Synthetic oligonucleotide"
ggtgtagtgggtttggttaagttggtttggtagagagggtgagatgtgtataagagacag

SEQ ID NO: 42 - DNA, 60 bp, Artificial Sequence
  source: /note="Description of Artificial Sequence: Synthetic oligonucleotide"
ggtgtagtgggtttggtataataatattggtagagagggtgagatgtgtataagagacag

SEQ ID NO: 43 - DNA, 60 bp, Artificial Sequence
  source: /note="Description of Artificial Sequence: Synthetic oligonucleotide"
ggtgtagtgggtttggaaggtatgagttggtagagagggtgagatgtgtataagagacag

SEQ ID NO: 44 - DNA, 60 bp, Artificial Sequence
  source: /note="Description of Artificial Sequence: Synthetic oligonucleotide"
ggtgtagtgggtttggaggattataagtggtagagagggtgagatgtgtataagagacag

SEQ ID NO: 45 - DNA, 60 bp, Artificial Sequence
  source: /note="Description of Artificial Sequence: Synthetic oligonucleotide"
ggtgtagtgggtttggagagttaggtttggtagagagggtgagatgtgtataagagacag

SEQ ID NO: 46 - DNA, 60 bp, Artificial Sequence
  source: /note="Description of Artificial Sequence: Synthetic oligonucleotide"
ggtgtagtgggtttggatggatagtattggtagagagggtgagatgtgtataagagacag

SEQ ID NO: 47 - DNA, 60 bp, Artificial Sequence
  source: /note="Description of Artificial Sequence: Synthetic oligonucleotide"
ggtgtagtgggtttggatattatgttgtggtagagagggtgagatgtgtataagagacag

SEQ ID NO: 48 - DNA, 60 bp, Artificial Sequence
  source: /note="Description of Artificial Sequence: Synthetic oligonucleotide"
ggtgtagtgggtttggggtggagatagtggtagagagggtgagatgtgtataagagacag

SEQ ID NO: 49 - DNA, 60 bp, Artificial Sequence
  source: /note="Description of Artificial Sequence: Synthetic oligonucleotide"
ggtgtagtgggtttggtggtggtagtgtggtagagagggtgagatgtgtataagagacag

SEQ ID NO: 50 - DNA, 60 bp, Artificial Sequence
  source: /note="Description of Artificial Sequence: Synthetic oligonucleotide"
ggtgtagtgggtttggaggtgagaagttggtagagagggtgagatgtgtataagagacag

SEQ ID NO: 51 - DNA, 60 bp, Artificial Sequence
  source: /note="Description of Artificial Sequence: Synthetic oligonucleotide"
ggtgtagtgggtttggtaggaggttgttggtagagagggtgagatgtgtataagagacag

SEQ ID NO: 52 - DNA, 60 bp, Artificial Sequence
  source: /note="Description of Artificial Sequence: Synthetic oligonucleotide"
ggtgtagtgggtttggtgtataggtattggtagagagggtgagatgtgtataagagacag

SEQ ID NO: 53 - DNA, 60 bp, Artificial Sequence
  source: /note="Description of Artificial Sequence: Synthetic oligonucleotide"
ggtgtagtgggtttggtgttatgtagatggtagagagggtgagatgtgtataagagacag

SEQ ID NO: 54 - DNA, 60 bp, Artificial Sequence
  source: /note="Description of Artificial Sequence: Synthetic oligonucleotide"
ggtgtagtgggtttggtggaaggtatgtggtagagagggtgagatgtgtataagagacag

SEQ ID NO: 55 - DNA, 60 bp, Artificial Sequence
  source: /note="Description of Artificial Sequence: Synthetic oligonucleotide"
ggtgtagtgggtttggaatgtaaggagtggtagagagggtgagatgtgtataagagacag

SEQ ID NO: 56 - DNA, 60 bp, Artificial Sequence
  source: /note="Description of Artificial Sequence: Synthetic oligonucleotide"
ggtgtagtgggtttgggttatgttaagtggtagagagggtgagatgtgtataagagacag

SEQ ID NO: 57 - DNA, 60 bp, Artificial Sequence
  source: /note="Description of Artificial Sequence: Synthetic oligonucleotide"
ggtgtagtgggtttggtgttataggtgtggtagagagggtgagatgtgtataagagacag

SEQ ID NO: 58 - DNA, 60 bp, Artificial Sequence
  source: /note="Description of Artificial Sequence: Synthetic oligonucleotide"
ggtgtagtgggtttggaaggagaattgtggtagagagggtgagatgtgtataagagacag

SEQ ID NO: 59 - DNA, 60 bp, Artificial Sequence
  source: /note="Description of Artificial Sequence: Synthetic oligonucleotide"
ggtgtagtgggtttggagaggtggaagtggtagagagggtgagatgtgtataagagacag

SEQ ID NO: 60 - DNA, 60 bp, Artificial Sequence
  source: /note="Description of Artificial Sequence: Synthetic oligonucleotide"
ggtgtagtgggtttgggattaggtgtatggtagagagggtgagatgtgtataagagacag

SEQ ID NO: 61 - DNA, 60 bp, Artificial Sequence
  source: /note="Description of Artificial Sequence: Synthetic oligonucleotide"
ggtgtagtgggtttggattatataagatggtagagagggtgagatgtgtataagagacag

SEQ ID NO: 62 - DNA, 60 bp, Artificial Sequence
  source: /note="Description of Artificial Sequence: Synthetic oligonucleotide"
ggtgtagtgggtttgggagaatatggttggtagagagggtgagatgtgtataagagacag

SEQ ID NO: 63 - DNA, 60 bp, Artificial Sequence
  source: /note="Description of Artificial Sequence: Synthetic oligonucleotide"
ggtgtagtgggtttggggattgagaggtggtagagagggtgagatgtgtataagagacag

SEQ ID NO: 64 - DNA, 60 bp, Artificial Sequence
  source: /note="Description of Artificial Sequence: Synthetic oligonucleotide"
ggtgtagtgggtttggattatggtggttggtagagagggtgagatgtgtataagagacag

SEQ ID NO: 65 - DNA, 60 bp, Artificial Sequence
  source: /note="Description of Artificial Sequence: Synthetic oligonucleotide"
ggtgtagtgggtttgggaaggaagttatggtagagagggtgagatgtgtataagagacag

SEQ ID NO: 66 - DNA, 60 bp, Artificial Sequence
  source: /note="Description of Artificial Sequence: Synthetic oligonucleotide"
ggtgtagtgggtttgggaatatgtaagtggtagagagggtgagatgtgtataagagacag

SEQ ID NO: 67 - DNA, 60 bp, Artificial Sequence
  source: /note="Description of Artificial Sequence: Synthetic oligonucleotide"
ggtgtagtgggtttggtagttaatatttggtagagagggtgagatgtgtataagagacag

SEQ ID NO: 68 - DNA, 60 bp, Artificial Sequence
  source: /note="Description of Artificial Sequence: Synthetic oligonucleotide"
ggtgtagtgggtttggtgaatgaatagtggtagagagggtgagatgtgtataagagacag

SEQ ID NO: 69 - DNA, 60 bp, Artificial Sequence
  source: /note="Description of Artificial Sequence: Synthetic oligonucleotide"
ggtgtagtgggtttggaggatggattatggtagagagggtgagatgtgtataagagacag

SEQ ID NO: 70 - DNA, 60 bp, Artificial Sequence
  source: /note="Description of Artificial Sequence: Synthetic oligonucleotide"
ggtgtagtgggtttggaagtgtatagatggtagagagggtgagatgtgtataagagacag

SEQ ID NO: 71 - DNA, 60 bp, Artificial Sequence
  source: /note="Description of Artificial Sequence: Synthetic oligonucleotide"
ggtgtagtgggtttgggaggttgaagatggtagagagggtgagatgtgtataagagacag

SEQ ID NO: 72 - DNA, 60 bp, Artificial Sequence
  source: /note="Description of Artificial Sequence: Synthetic oligonucleotide"
ggtgtagtgggtttggtgtgtaataggtggtagagagggtgagatgtgtataagagacag

SEQ ID NO: 73 - DNA, 60 bp, Artificial Sequence
  source: /note="Description of Artificial Sequence: Synthetic oligonucleotide"
ggtgtagtgggtttggttgattagagatggtagagagggtgagatgtgtataagagacag

SEQ ID NO: 74 - DNA, 60 bp, Artificial Sequence
  source: /note="Description of Artificial Sequence: Synthetic oligonucleotide"
ggtgtagtgggtttggtatgtgtgtggtggtagagagggtgagatgtgtataagagacag

SEQ ID NO: 75 - DNA, 60 bp, Artificial Sequence
  source: /note="Description of Artificial Sequence: Synthetic oligonucleotide"
ggtgtagtgggtttgggagatgagaattggtagagagggtgagatgtgtataagagacag

SEQ ID NO: 76 - DNA, 60 bp, Artificial Sequence
  source: /note="Description of Artificial Sequence: Synthetic oligonucleotide"
ggtgtagtgggtttggtggtgaagtgatggtagagagggtgagatgtgtataagagacag

SEQ ID NO: 77 - DNA, 60 bp, Artificial Sequence
  source: /note="Description of Artificial Sequence: Synthetic oligonucleotide"
ggtgtagtgggtttgggtggtaggatgtggtagagagggtgagatgtgtataagagacag

SEQ ID NO: 78 - DNA, 60 bp, Artificial Sequence
  source: /note="Description of Artificial Sequence: Synthetic oligonucleotide"
ggtgtagtgggtttggtgtaggtgatatggtagagagggtgagatgtgtataagagacag

SEQ ID NO: 79 - DNA, 60 bp, Artificial Sequence
  source: /note="Description of Artificial Sequence: Synthetic oligonucleotide"
ggtgtagtgggtttgggtaaggtgtgatggtagagagggtgagatgtgtataagagacag

SEQ ID NO: 80 - DNA, 60 bp, Artificial Sequence
  source: /note="Description of Artificial Sequence: Synthetic oligonucleotide"
ggtgtagtgggtttggagaagagagtgtggtagagagggtgagatgtgtataagagacag

SEQ ID NO: 81 - DNA, 60 bp, Artificial Sequence
  source: /note="Description of Artificial Sequence: Synthetic oligonucleotide"
ggtgtagtgggtttggggatgttgtattggtagagagggtgagatgtgtataagagacag

SEQ ID NO: 82 - DNA, 60 bp, Artificial Sequence
  source: /note="Description of Artificial Sequence: Synthetic oligonucleotide"
ggtgtagtgggtttggaagttatataatggtagagagggtgagatgtgtataagagacag

SEQ ID NO: 83 - DNA, 60 bp, Artificial Sequence
  source: /note="Description of Artificial Sequence: Synthetic oligonucleotide"
ggtgtagtgggtttggtggaattaagttggtagagagggtgagatgtgtataagagacag

SEQ ID NO: 84 - DNA, 60 bp, Artificial Sequence
  source: /note="Description of Artificial Sequence: Synthetic oligonucleotide"
ggtgtagtgggtttggtaatgagaggatggtagagagggtgagatgtgtataagagacag

SEQ ID NO: 85 - DNA, 60 bp, Artificial Sequence
  source: /note="Description of Artificial Sequence: Synthetic oligonucleotide"
ggtgtagtgggtttggataattgatggtggtagagagggtgagatgtgtataagagacag

SEQ ID NO: 86 - DNA, 60 bp, Artificial Sequence
  source: /note="Description of Artificial Sequence: Synthetic oligonucleotide"
ggtgtagtgggtttggtgtgaagagtatggtagagagggtgagatgtgtataagagacag

SEQ ID NO: 87 - DNA, 60 bp, Artificial Sequence
  source: /note="Description of Artificial Sequence: Synthetic oligonucleotide"
ggtgtagtgggtttgggatgaatatgttggtagagagggtgagatgtgtataagagacag

SEQ ID NO: 88 - DNA, 60 bp, Artificial Sequence
  source: /note="Description of Artificial Sequence: Synthetic oligonucleotide"
ggtgtagtgggtttggtgaggatagattggtagagagggtgagatgtgtataagagacag

SEQ ID NO: 89 - DNA, 60 bp, Artificial Sequence
  source: /note="Description of Artificial Sequence: Synthetic oligonucleotide"
ggtgtagtgggtttggattaattagagtggtagagagggtgagatgtgtataagagacag

SEQ ID NO: 90 - DNA, 60 bp, Artificial Sequence
  source: /note="Description of Artificial Sequence: Synthetic oligonucleotide"
ggtgtagtgggtttggggagagatggatggtagagagggtgagatgtgtataagagacag

SEQ ID NO: 91 - DNA, 60 bp, Artificial Sequence
  source: /note="Description of Artificial Sequence: Synthetic oligonucleotide"
ggtgtagtgggtttggtaattgaggaatggtagagagggtgagatgtgtataagagacag

SEQ ID NO: 92 - DNA, 60 bp, Artificial Sequence
  source: /note="Description of Artificial Sequence: Synthetic oligonucleotide"
ggtgtagtgggtttggttggaattaattggtagagagggtgagatgtgtataagagacag

SEQ ID NO: 93 - DNA, 60 bp, Artificial Sequence
  source: /note="Description of Artificial Sequence: Synthetic oligonucleotide"
ggtgtagtgggtttggaatgttattgttggtagagagggtgagatgtgtataagagacag

SEQ ID NO: 94 - DNA, 60 bp, Artificial Sequence
  source: /note="Description of Artificial Sequence: Synthetic oligonucleotide"
ggtgtagtgggtttgggtagttattagtggtagagagggtgagatgtgtataagagacag

SEQ ID NO: 95 - DNA, 60 bp, Artificial Sequence
  source: /note="Description of Artificial Sequence: Synthetic oligonucleotide"
ggtgtagtgggtttggtatattgtgagtggtagagagggtgagatgtgtataagagacag

SEQ ID NO: 96 - DNA, 60 bp, Artificial Sequence
  source: /note="Description of Artificial Sequence: Synthetic oligonucleotide"
ggtgtagtgggtttgggtgtaggatagtggtagagagggtgagatgtgtataagagacag

SEQ ID NO: 97 - DNA, 60 bp, Artificial Sequence
  source: /note="Description of Artificial Sequence: Synthetic oligonucleotide"
ggtgtagtgggtttggagagaagttggtggtagagagggtgagatgtgtataagagacag

SEQ ID NO: 98 - DNA, 37 bp, Artificial Sequence
  source: /note="Description of Artificial Sequence: Synthetic primer"
  modified_base (29)..(37): a, c, t, g, unknown or other
ggagttcagacgtgtgctcttccgatctnnnnnnnnn

SEQ ID NO: 99 - DNA, 68 bp, Artificial Sequence
  source: /note="Description of Artificial Sequence: Synthetic primer"
caagcagaagacggcatacgagatcaagatgccggtgactggagttcagacgtgtgctcttccgatct

SEQ ID NO: 100 - DNA, 68 bp, Artificial Sequence
  source: /note="Description of Artificial Sequence: Synthetic primer"
caagcagaagacggcatacgagataacgtctagtgtgactggagttcagacgtgtgctcttccgatct

SEQ ID NO: 101 - DNA, 68 bp, Artificial Sequence
  source: /note="Description of Artificial Sequence: Synthetic primer"
caagcagaagacggcatacgagataggtatactcgtgactggagttcagacgtgtgctcttccgatct

SEQ ID NO: 102 - DNA, 68 bp, Artificial Sequence
  source: /note="Description of Artificial Sequence: Synthetic primer"
caagcagaagacggcatacgagatttcataggacgtgactggagttcagacgtgtgctcttccgatct

SEQ ID NO: 103 - DNA, 68 bp, Artificial Sequence
  source: /note="Description of Artificial Sequence: Synthetic primer"
caagcagaagacggcatacgagatggaggcctccgtgactggagttcagacgtgtgctcttccgatct

SEQ ID NO: 104 - DNA, 68 bp, Artificial Sequence
  source: /note="Description of Artificial Sequence: Synthetic primer"
caagcagaagacggcatacgagatttcaatataagtgactggagttcagacgtgtgctcttccgatct

SEQ ID NO: 105 - DNA, 68 bp, Artificial Sequence
  source: /note="Description of Artificial Sequence: Synthetic primer"
caagcagaagacggcatacgagatacgtcatatagtgactggagttcagacgtgtgctcttccgatct

SEQ ID NO: 106 - DNA, 68 bp, Artificial Sequence
  source: /note="Description of Artificial Sequence: Synthetic primer"
caagcagaagacggcatacgagatttgaccaggagtgactggagttcagacgtgtgctcttccgatct

SEQ ID NO: 107 - DNA, 68 bp, Artificial Sequence
  source: /note="Description of Artificial Sequence: Synthetic primer"
caagcagaagacggcatacgagatcggttgcgcggtgactggagttcagacgtgtgctcttccgatct

SEQ ID NO: 108 - DNA, 68 bp, Artificial Sequence
  source: /note="Description of Artificial Sequence: Synthetic primer"
caagcagaagacggcatacgagatcaaggaggtcgtgactggagttcagacgtgtgctcttccgatct

SEQ ID NO: 109 - DNA, 68 bp, Artificial Sequence
  source: /note="Description of Artificial Sequence: Synthetic primer"
caagcagaagacggcatacgagatttacgatgaagtgactggagttcagacgtgtgctcttccgatct

SEQ ID NO: 110 - DNA, 68 bp, Artificial Sequence
  source: /note="Description of Artificial Sequence: Synthetic primer"
caagcagaagacggcatacgagatttgctggcatgtgactggagttcagacgtgtgctcttccgatct

SEQ ID NO: 111 - DNA, 68 bp, Artificial Sequence
  source: /note="Description of Artificial Sequence: Synthetic primer"
caagcagaagacggcatacgagataatactcttcgtgactggagttcagacgtgtgctcttccgatct

SEQ ID NO: 112 - DNA, 68 bp, Artificial Sequence
  source: /note="Description of Artificial Sequence: Synthetic primer"
caagcagaagacggcatacgagatccaactaaccgtgactggagttcagacgtgtgctcttccgatct

SEQ ID NO: 113 - DNA, 68 bp, Artificial Sequence
  source: /note="Description of Artificial Sequence: Synthetic primer"
caagcagaagacggcatacgagattatcctcaatgtgactggagttcagacgtgtgctcttccgatct

SEQ ID NO: 114 - DNA, 68 bp, Artificial Sequence
  source: /note="Description of Artificial Sequence: Synthetic primer"
caagcagaagacggcatacgagatgccgtcgcgtgtgactggagttcagacgtgtgctcttccgatct

SEQ ID NO: 115 - DNA, 68 bp, Artificial Sequence
  source: /note="Description of Artificial Sequence: Synthetic primer"
caagcagaagacggcatacgagatccgctgcttcgtgactggagttcagacgtgtgctcttccgatct

SEQ ID NO: 116 - DNA, 68 bp, Artificial Sequence
  source: /note="Description of Artificial Sequence: Synthetic primer"
caagcagaagacggcatacgagattgaccgaatcgtgactggagttcagacgtgtgctcttccgatct

SEQ ID NO: 117 - DNA, 68 bp, Artificial Sequence
  source: /note="Description of Artificial Sequence: Synthetic primer"
caagcagaagacggcatacgagatgtctccagaggtgactggagttcagacgtgtgctcttccgatct

SEQ ID NO: 118 - DNA, 68 bp, Artificial Sequence
  source: /note="Description of Artificial Sequence: Synthetic primer"
caagcagaagacggcatacgagataatgctagtcgtgactggagttcagacgtgtgctcttccgatct

SEQ ID NO: 119 - DNA, 68 bp, Artificial Sequence
  source: /note="Description of Artificial Sequence: Synthetic primer"
caagcagaagacggcatacgagatgacgacctgcgtgactggagttcagacgtgtgctcttccgatct

SEQ ID NO: 120 - DNA, 68 bp, Artificial Sequence
  source: /note="Description of Artificial Sequence: Synthetic primer"
caagcagaagacggcatacgagatagagccagccgtgactggagttcagacgtgtgctcttccgatct

SEQ ID NO: 121 - DNA, 68 bp, Artificial Sequence
  source: /note="Description of Artificial Sequence: Synthetic primer"
caagcagaagacggcatacgagatccaggccgcagtgactggagttcagacgtgtgctcttccgatct

SEQ ID NO: 122 - DNA, 68 bp, Artificial Sequence
  source: /note="Description of Artificial Sequence: Synthetic primer"
caagcagaagacggcatacgagatcaggtatggagtgactggagttcagacgtgtgctcttccgatct

SEQ ID NO: 123 - DNA, 55 bp, Artificial Sequence
  source: /note="Description of Artificial Sequence: Synthetic primer"
aatgatacggcgaccaccgagatctacacgtatcatcgaggtgtagtgggtttgg

SEQ ID NO: 124 - DNA, 55 bp, Artificial Sequence
  source: /note="Description of Artificial Sequence: Synthetic primer"
aatgatacggcgaccaccgagatctacacccgcgattatggtgtagtgggtttgg

SEQ ID NO: 125 - DNA, 55 bp, Artificial Sequence
  source: /note="Description of Artificial Sequence: Synthetic primer"
aatgatacggcgaccaccgagatctacacattcaggtacggtgtagtgggtttgg

SEQ ID NO: 126 - DNA, 55 bp, Artificial Sequence
  source: /note="Description of Artificial Sequence: Synthetic primer"
aatgatacggcgaccaccgagatctacacatggaattggggtgtagtgggtttgg

SEQ ID NO: 127 - DNA, 55 bp, Artificial Sequence
  source: /note="Description of Artificial Sequence: Synthetic primer"
aatgatacggcgaccaccgagatctacacgacgaagcgtggtgtagtgggtttgg

SEQ ID NO: 128 - DNA, 55 bp, Artificial Sequence
  source: /note="Description of Artificial Sequence: Synthetic primer"
aatgatacggcgaccaccgagatctacaccttgcagtagggtgtagtgggtttgg

SEQ ID NO: 129 - DNA, 55 bp, Artificial Sequence
  source: /note="Description of Artificial Sequence: Synthetic primer"
aatgatacggcgaccaccgagatctacaccttggtaatgggtgtagtgggtttgg

SEQ ID NO: 130 - DNA, 55 bp, Artificial Sequence
  source: /note="Description of Artificial Sequence: Synthetic primer"
aatgatacggcgaccaccgagatctacaccaagtcgaccggtgtagtgggtttgg

SEQ ID NO: 131 - DNA, 33 bp, Artificial Sequence
  source: /note="Description of Artificial Sequence: Synthetic primer"
tggtagagagggtgagatgtgtataagagatag

SEQ ID NO: 132 - DNA, 33 bp, Artificial Sequence
  source: /note="Description of Artificial Sequence: Synthetic primer"
ctatctcttatacacatctcaccctctctacca